European Patent Application EP 4 129 286 A1, published February 8, 2023. Title: DDR2 MUTATIONS AS TARGETABLE FEATURES OF MELANOMA OR BASAL CELL CARCINOMA. Applicant: JONES, DANIEL M. WANG, YONGBAO BILLOUIN-FRAZIER, SHERE WINDHAM, JUSTIN. Application PCT/US2013/077832. The sequence listing filed with the application follows.

SEQUENCE LISTING (169 sequences)

SEQ ID NO: 1 - DNA, 21 bp, Artificial Sequence
  Description of Artificial Sequence: Synthetic primer
tccagttccaacaccatcttc

SEQ ID NO: 2 - DNA, 23 bp, Artificial Sequence
  Description of Artificial Sequence: Synthetic primer
tttctctttggtttctcttggtc

SEQ ID NO: 3 - DNA, 20 bp, Artificial Sequence
  Description of Artificial Sequence: Synthetic primer
cccaaccctcacctctcaag

SEQ ID NO: 4 - DNA, 20 bp, Artificial Sequence
  Description of Artificial Sequence: Synthetic primer
ccagtggaacctgatgacct

SEQ ID NO: 5 - DNA, 18 bp, Artificial Sequence
  Description of Artificial Sequence: Synthetic primer
ccatgcaggaggtcatgg

SEQ ID NO: 6 - DNA, 24 bp, Artificial Sequence
  Description of Artificial Sequence: Synthetic primer
cactcattctcttctctctcctca

SEQ ID NO: 7 - DNA, 21 bp, Artificial Sequence
  Description of Artificial Sequence: Synthetic primer
ccattgtagccagatttgtcc

SEQ ID NO: 8 - DNA, 20 bp, Artificial Sequence
  Description of Artificial Sequence: Synthetic primer
cttggctgtgtttcctttgc

SEQ ID NO: 9 - DNA, 19 bp, Artificial Sequence
  Description of Artificial Sequence: Synthetic primer
ctcttctcctggcctgagc

SEQ ID NO: 10 - DNA, 20 bp, Artificial Sequence
  Description of Artificial Sequence: Synthetic primer
cccagacccatgaataccac

SEQ ID NO: 11 - DNA, 22 bp, Artificial Sequence
  Description of Artificial Sequence: Synthetic primer
tcacatgcctctttctctacca

SEQ ID NO: 12 - DNA, 20 bp, Artificial Sequence
  Description of Artificial Sequence: Synthetic primer
cagtgctacttccgctctga

SEQ ID NO: 13 - DNA, 18 bp, Artificial Sequence
  Description of Artificial Sequence: Synthetic primer
cccagtgctcggtttgtc

SEQ ID NO: 14 - DNA, 21 bp, Artificial Sequence
  Description of Artificial Sequence: Synthetic primer
gctctgactcacccttgtttt

SEQ ID NO: 15 - DNA, 20 bp, Artificial Sequence
  Description of Artificial Sequence: Synthetic primer
ccttctctccctggtcacag

SEQ ID NO: 16 - DNA, 19 bp, Artificial Sequence
  Description of Artificial Sequence: Synthetic primer
ggatcctgattggctgctt

SEQ ID NO: 17 - DNA, 21 bp, Artificial Sequence
  Description of Artificial Sequence: Synthetic primer
tctccttgctcttctcttcca

SEQ ID NO: 18 - DNA, 20 bp, Artificial Sequence
  Description of Artificial Sequence: Synthetic primer
accgctcctcatcacctagt

SEQ ID NO: 19 - DNA, 19 bp, Artificial Sequence
  Description of Artificial Sequence: Synthetic primer
ctcgttgcccttgtcttcc

SEQ ID NO: 20 - DNA, 18 bp, Artificial Sequence
  Description of Artificial Sequence: Synthetic primer
gagggggtgccccactat

SEQ ID NO: 21 - DNA, 18 bp, Artificial Sequence
  Description of Artificial Sequence: Synthetic primer
agtgcctgccgtcaccat

SEQ ID NO: 22 - DNA, 25 bp, Artificial Sequence
  Description of Artificial Sequence: Synthetic primer
tgatgctgagactagatgacttttg

SEQ ID NO: 23 - DNA, 21 bp, Artificial Sequence
  Description of Artificial Sequence: Synthetic primer
gggaatggaaaaattcaaaga

SEQ ID NO: 24 - DNA, 26 bp, Artificial Sequence
  Description of Artificial Sequence: Synthetic primer
tttatctatgtctgtatcctcccaag

SEQ ID NO: 25 - DNA, 26 bp, Artificial Sequence
  Description of Artificial Sequence: Synthetic primer
ccatctattagctgtgtgtatcactg

SEQ ID NO: 26 - DNA, 26 bp, Artificial Sequence
  Description of Artificial Sequence: Synthetic primer
ccttctgtcttcttgtctatttcctc

SEQ ID NO: 27 - DNA, 23 bp, Artificial Sequence
  Description of Artificial Sequence: Synthetic primer
tctcttaattttgttcaccgaga

SEQ ID NO: 28 - DNA, 20 bp, Artificial Sequence
  Description of Artificial Sequence: Synthetic primer
ctttggaatgagcaggaacc

SEQ ID NO: 29 - DNA, 25 bp, Artificial Sequence
  Description of Artificial Sequence: Synthetic primer
tgatttcccattcttttctttactt

SEQ ID NO: 30 - DNA, 22 bp, Artificial Sequence
  Description of Artificial Sequence: Synthetic primer
tttgtgggagactttcaccttt

SEQ ID NO: 31 - DNA, 24 bp, Artificial Sequence
  Description of Artificial Sequence: Synthetic primer
tttcctttatttttgttcccaaag

SEQ ID NO: 32 - DNA, 21 bp, Artificial Sequence
  Description of Artificial Sequence: Synthetic primer
gctgctggagaagagatacga

SEQ ID NO: 33 - DNA, 22 bp, Artificial Sequence
  Description of Artificial Sequence: Synthetic primer
tctgtttggcttgacttgactt

SEQ ID NO: 34 - DNA, 20 bp, Artificial Sequence
  Description of Artificial Sequence: Synthetic primer
gacgggactcgagtgatgat

SEQ ID NO: 35 - DNA, 20 bp, Artificial Sequence
  Description of Artificial Sequence: Synthetic primer
gcgatcgtaagtcgagttgg

SEQ ID NO: 36 - DNA, 19 bp, Artificial Sequence
  Description of Artificial Sequence: Synthetic primer
cccaccacatcatcctcac

SEQ ID NO: 37 - DNA, 20 bp, Artificial Sequence
  Description of Artificial Sequence: Synthetic primer
tgtgttgcctcctgtcactc

SEQ ID NO: 38 - DNA, 18 bp, Artificial Sequence
  Description of Artificial Sequence: Synthetic primer
tggggaactcctccacag

SEQ ID NO: 39 - DNA, 23 bp, Artificial Sequence
  Description of Artificial Sequence: Synthetic primer
aagggaatcaaagaatcaactca

SEQ ID NO: 40 - DNA, 18 bp, Artificial Sequence
  Description of Artificial Sequence: Synthetic primer
gctcggagcattttcaca

SEQ ID NO: 41 - DNA, 25 bp, Artificial Sequence
  Description of Artificial Sequence: Synthetic primer
ggaaaattcaaaatgtagaccacag

SEQ ID NO: 42 - DNA, 27 bp, Artificial Sequence
  Description of Artificial Sequence: Synthetic primer
catgtattcagtgatcatacagagagg

SEQ ID NO: 43 - DNA, 21 bp, Artificial Sequence
  Description of Artificial Sequence: Synthetic primer
agaaggaagacctggcttgtt

SEQ ID NO: 44 - DNA, 26 bp, Artificial Sequence
  Description of Artificial Sequence: Synthetic primer
tgtgtagttcttacccactaaacagt

SEQ ID NO: 45 - DNA, 20 bp, Artificial Sequence
  Description of Artificial Sequence: Synthetic primer
gccctggatccggtaatagt

SEQ ID NO: 46 - DNA, 21 bp, Artificial Sequence
  Description of Artificial Sequence: Synthetic primer
cagggctttaaaatgctgaga

SEQ ID NO: 47 - DNA, 20 bp, Artificial Sequence
  Description of Artificial Sequence: Synthetic primer
tctgacagctgggaataggg

SEQ ID NO: 48 - DNA, 20 bp, Artificial Sequence
  Description of Artificial Sequence: Synthetic primer
ccattcatccccaacagttc

SEQ ID NO: 49 - DNA, 20 bp, Artificial Sequence
  Description of Artificial Sequence: Synthetic primer
gcagaaggtggatttcttgg

SEQ ID NO: 50 - DNA, 20 bp, Artificial Sequence
  Description of Artificial Sequence: Synthetic primer
aggacctgagccgtaggaac

SEQ ID NO: 51 - DNA, 20 bp, Artificial Sequence
  Description of Artificial Sequence: Synthetic primer
tccaattctttgtcccactg

SEQ ID NO: 52 - DNA, 23 bp, Artificial Sequence
  Description of Artificial Sequence: Synthetic primer
tgtcacaatgtcaccacattaca

SEQ ID NO: 53 - DNA, 20 bp, Artificial Sequence
  Description of Artificial Sequence: Synthetic primer
gacccactccatcgagattt

SEQ ID NO: 54 - DNA, 21 bp, Artificial Sequence
  Description of Artificial Sequence: Synthetic primer
tcagtggaaaaatagcctcaa

SEQ ID NO: 55 - DNA, 43 bp, Artificial Sequence
  Description of Artificial Sequence: Synthetic primer
tgtaaaacgacggccagttgagaattgtactcattcatgttgg

SEQ ID NO: 56 - DNA, 38 bp, Artificial Sequence
  Description of Artificial Sequence: Synthetic primer
caggaaacagctatgaccgtagtccctcttggcagctt

SEQ ID NO: 57 - DNA, 44 bp, Artificial Sequence
  Description of Artificial Sequence: Synthetic primer
tgtaaaacgacggccagttcttattccttgttcaatattcagtg

SEQ ID NO: 58 - DNA, 38 bp, Artificial Sequence
  Description of Artificial Sequence: Synthetic primer
caggaaacagctatgacccccctagggtcaggaatctg

SEQ ID NO: 59 - DNA, 37 bp, Artificial Sequence
  Description of Artificial Sequence: Synthetic primer
tgtaaaacgacggccagtcagctgcttgcctgtgaac

SEQ ID NO: 60 - DNA, 41 bp, Artificial Sequence
  Description of Artificial Sequence: Synthetic primer
caggaaacagctatgacccacacagaaaacctgtacccttc

SEQ ID NO: 61 - DNA, 38 bp, Artificial Sequence
  Description of Artificial Sequence: Synthetic primer
tgtaaaacgacggccagtgtggtggggtgaagaaaagt

SEQ ID NO: 62 - DNA, 38 bp, Artificial Sequence
  Description of Artificial Sequence: Synthetic primer
caggaaacagctatgacctccctttctgatttgattgc

SEQ ID NO: 63 - DNA, 38 bp, Artificial Sequence
  Description of Artificial Sequence: Synthetic primer
tgtaaaacgacggccagtcgctgtgcaagcttataccc

SEQ ID NO: 64 - DNA, 41 bp, Artificial Sequence
  Description of Artificial Sequence: Synthetic primer
caggaaacagctatgaccttgattgattattgatcccaaga

SEQ ID NO: 65 - DNA, 38 bp, Artificial Sequence
  Description of Artificial Sequence: Synthetic primer
tgtaaaacgacggccagtgagtgaagatgccgggtaaa

SEQ ID NO: 66 - DNA, 38 bp, Artificial Sequence
  Description of Artificial Sequence: Synthetic primer
caggaaacagctatgacctgaactggcatcagcctaga

SEQ ID NO: 67 - DNA, 38 bp, Artificial Sequence
  Description of Artificial Sequence: Synthetic primer
tgtaaaacgacggccagttactgagttggctggcactg

SEQ ID NO: 68 - DNA, 38 bp, Artificial Sequence
  Description of Artificial Sequence: Synthetic primer
caggaaacagctatgacctgagaagttctgggcatgtg

SEQ ID NO: 69 - DNA, 43 bp, Artificial Sequence
  Description of Artificial Sequence: Synthetic primer
tgtaaaacgacggccagttcactaaattgatcttgtaatgtgc

SEQ ID NO: 70 - DNA, 38 bp, Artificial Sequence
  Description of Artificial Sequence: Synthetic primer
caggaaacagctatgaccccagggctactcttcatcca

SEQ ID NO: 71 - DNA, 38 bp, Artificial Sequence
  Description of Artificial Sequence: Synthetic primer
tgtaaaacgacggccagtaggaacagggtctacctcca

SEQ ID NO: 72 - DNA, 40 bp, Artificial Sequence
  Description of Artificial Sequence: Synthetic primer
caggaaacagctatgaccaaatgtttgcaatttgcctttt

SEQ ID NO: 73 - DNA, 41 bp, Artificial Sequence
  Description of Artificial Sequence: Synthetic primer
tgtaaaacgacggccagttgggagagctgagtttaagaaga

SEQ ID NO: 74 - DNA, 44 bp, Artificial Sequence
  Description of Artificial Sequence: Synthetic primer
caggaaacagctatgaccgcagagactaaaaatagatgcaatga

SEQ ID NO: 75 - DNA, 38 bp, Artificial Sequence
  Description of Artificial Sequence: Synthetic primer
tgtaaaacgacggccagtgccctcctctcagagttcct

SEQ ID NO: 76 - DNA, 38 bp, Artificial Sequence
  Description of Artificial Sequence: Synthetic primer
caggaaacagctatgaccgtgaatccacctctggaagg

SEQ ID NO: 77 - DNA, 38 bp, Artificial Sequence
  Description of Artificial Sequence: Synthetic primer
tgtaaaacgacggccagtggaaatgcccagcaagagta

SEQ ID NO: 78 - DNA, 38 bp, Artificial Sequence
  Description of Artificial Sequence: Synthetic primer
caggaaacagctatgaccgctcactgaccttcccatct

SEQ ID NO: 79 - DNA, 38 bp, Artificial Sequence
  Description of Artificial Sequence: Synthetic primer
tgtaaaacgacggccagtataggccttggtgtgcattc

SEQ ID NO: 80 - DNA, 37 bp, Artificial Sequence
  Description of Artificial Sequence: Synthetic primer
caggaaacagctatgaccactgacttcccccaccatc

SEQ ID NO: 81 - DNA, 40 bp, Artificial Sequence
  Description of Artificial Sequence: Synthetic primer
tgtaaaacgacggccagtgaatgttgagctttcaacccta

SEQ ID NO: 82 - DNA, 38 bp, Artificial Sequence
  Description of Artificial Sequence: Synthetic primer
caggaaacagctatgaccagcccacaagccagttgtta

SEQ ID NO: 83 - DNA, 38 bp, Artificial Sequence
  Description of Artificial Sequence: Synthetic primer
tgtaaaacgacggccagtagaattccttgcctgtggtg

SEQ ID NO: 84 - DNA, 41 bp, Artificial Sequence
  Description of Artificial Sequence: Synthetic primer
caggaaacagctatgaccagtgacaaagactaacacctgga

SEQ ID NO: 85 - DNA, 39 bp, Artificial Sequence
  Description of Artificial Sequence: Synthetic primer
tgtaaaacgacggccagtcaaatcaaaccatgatgcaaa

SEQ ID NO: 86 - DNA, 38 bp, Artificial Sequence
  Description of Artificial Sequence: Synthetic primer
caggaaacagctatgacctgtccagatggagtggcata

SEQ ID NO: 87 - DNA, 18 bp, Artificial Sequence
  Description of Artificial Sequence: Synthetic primer
tgtaaaacgacggccagt

SEQ ID NO: 88 - DNA, 18 bp, Artificial Sequence
  Description of Artificial Sequence: Synthetic primer
caggaaacagctatgacc

SEQ ID NO: 89 - protein, 830 aa, Unknown
  Description of Unknown: DDR2 polypeptide
KAQVNPAICRYPLGMSGGQIPDEDITASSQWSESTAAKYGRLDSEEGDGAWCPEIPVEPDDLKEFLQIDLHTLHFITLVGTQGRHAGGHGIEFAPMYKINYSRDGTRWISWRNRHGKQVLDGNSNPYDIFLKDLEPPIVARFVRFIPVTDHSMNVCMRVELYGCVWLDGLVSYNAPAGQQFVLPGGSIIYLNDSVYDGAVGYSMTEGLGQLTDGVSGLDDFTQTHEYHVWPGYDYVGWRNESATNGYIEIMFEFDRIRNFTTMKVHCNNMFAKGVKIFKEVQCYFRSEASEWEPNAISFPLVLDDVNPSARFVTVPLHHRMASAIKCQYHFADTWMMFSEITFQSDAAMYNNSEALPTSPMAPTTYDPMLKVDDSNTRILIGCLVAIIFILLAIIVIILWRQFWQKMLEKASRRMLDDEMTVSLSLPSDSSMFNNNRSSSPSEQGSNSTYDRIFPLRPDYQEPSRLIRKLPEFAPGEEESGCSGVVKPVQPSGPEGVPHYAEADIVNLQGVTGGNTYSVPAVTMDLLSGKDVAVEEFPRKLLTFKEKLGEGQFGEVHLCEVEGMEKFKDKDFALDVSANQPVLVAVKMLRADANKNARNDFLKEIKIMSRLKDPNIIHLLSVCITDDPLCMITEYMENGDLNQFLSRHEPPNSSSSDVRTVSYTNLKFMATQIASGMKYLSSLNFVHRDLATRNCLVGKNYTIKIADFGMSRNLYSGDYYRIQGRAVLPIRWMSWESILLGKFTTASDVWAFGVTLWETFTFCQEQPYSQLSDEQVIENTGEFFRDQGRQTYLPQPAICPDSVYKLMLSCWRRDTKNRPSFQEIHLLLLQ

SEQ ID NO: 90 - protein, 847 aa, Unknown
  Description of Unknown: DDR1 polypeptide
KGHFDPAKCRYALGMQDRTIPDSDISASSSWSDSTAARHSRLESSDGDGAWCPAGSVFPKEEEYLQVDLQRLHLVALVGTQGRHAGGLGKEFSRSYRLRYSRDGRRWMGWKDRWGQEVISGNEDPEGVVLKDLGPPMVARLVRFYPRADRVMSVCLRVELYGCLWRDGLLSYTAPVGQTMYLSEAVYLNDSTYDGHTVGGLQYGGLGQLADGVVGLDDFRKSQELRVWPGYDYVGWSNHSFSSGYVEMEFEFDRLRAFQAMQVHCNNMHTLGARLPGGVECRFRRGPAMAWEGEPMRHNLGGNLGDPRARAVSVPLGGRVARFLQCRFLFAGPWLLFSEISFISDVVNNSSPALGGTFPPAPWWPPGPPPTNFSSLELEPRGQQPVAKAEGSPTAILIGCLVAIILLLLLIIALMLWRLHWRRLLSAERRVLEEELTVHLSVPGDTILINNRPGPREPPPYQEPRPRGNPPHSAPCVPNGSAYSGDYMEPEKPGAPLLPPPPQNSVPHYAEADIVTLQGVTGGNTYAVPALPPGAVGDGPPRVDFPRSRLRFKEKLGEGQFGEVHLCEVDSPQDLVSLDFPLNVRKGHPLLVAVKILRPDATKNARNDFLKEVKIMSRLKDPNIIRLLGVCVQDDPLCMITDYMENGDLNQFLSAHQLEDKAAEGAPGDGQAAQGPTISYPMLLHVAAQIASGMRYLATLNFVHRDLATRNCLVGENFTIKIADFGMSRNLYAGDYYRVQGRAVLPIRWMAWECILMGKFTTASDVWAFGVTLWEVLMLCRAQPFGQLTDEQVIENAGEFFRDQGRQVYLSRPPACPQGLYELMLRCWSRESEQRPPFSQLHRFLAE

SEQ ID NO: 91 - DNA, 20 bp, Unknown
  Description of Unknown: DDR2 oligonucleotide
tgggagaaggacagtttggg

SEQ ID NO: 92 - DNA, 20 bp, Unknown
  Description of Unknown: DDR2 oligonucleotide
tgggagaaggacagtktggg

SEQ ID NO: 93 - DNA, 20 bp, Unknown
  Description of Unknown: DDR2 oligonucleotide
tgggagaaggacagtgtggg

SEQ ID NO: 94 - DNA, 20 bp, Unknown
  Description of Unknown: DDR2 oligonucleotide
tgggagaaggacattttggg

SEQ ID NO: 95 - DNA, 20 bp, Unknown
  Description of Unknown: DDR2 oligonucleotide
tgggagagggacagtttggg

SEQ ID NO: 96 - DNA, 20 bp, Unknown
  Description of Unknown: DDR2 oligonucleotide
tgggagagggacaagttggg

SEQ ID NO: 97 - protein, 7 aa, Unknown
  Description of Unknown: DDR2 peptide
LGEGQFG

SEQ ID NO: 98 - DNA, 21 bp, Unknown
  Description of Unknown: DDR2 oligonucleotide
tgggagaaggacagtktgggg

SEQ ID NO: 99 - protein, 23 aa, Unknown
  Description of Unknown: DDR2 peptide
FKEKLGEGQFGEVHLCEVEGMEK

SEQ ID NO: 100 - protein, 21 aa, Unknown
  Description of Unknown: BRAF peptide
VGQRIGSGSFGTVYKGKWHGD

SEQ ID NO: 101 - protein, 23 aa, Unknown
  Description of Unknown: EGFR peptide
KIKVLGSGAFGTVYKGLWIPEGE

SEQ ID NO: 102 - protein, 23 aa, Unknown
  Description of Unknown: ERBB2 peptide
KVKVLGSGAFGTVYKGIWIPDGE

SEQ ID NO: 103 - protein, 19 aa, Unknown
  Description of Unknown: ABL1 peptide
MKHKLGGGQYGEVYEGVWK

SEQ ID NO: 104 - protein, 23 aa, Unknown
  Description of Unknown: ALK peptide
LIRGLGHGAFGEVYEGQVSGMPN

SEQ ID NO: 105 - protein, 23 aa, Unknown
  Description of Unknown: AKT1 peptide
YLKLLGKGTFGKVILVKEKATGR

SEQ ID NO: 106 - protein, 23 aa, Unknown
  Description of Unknown: MET peptide
FNEVIGRGHFGCVYHGTLLDNDG

SEQ ID NO: 107 - protein, 23 aa, Unknown
  Description of Unknown: FGFR1 peptide
LGKPLGEGCFGQVVLAEAIGLDK

SEQ ID NO: 108 - protein, 23 aa, Unknown
  Description of Unknown: FGFR2 peptide
LGKPLGEGCFGQVVLAEAIGIDK

SEQ ID NO: 109 - protein, 23 aa, Unknown
  Description of Unknown: FGFR3 peptide
LGKPLGEGCFGQVVLAEAIGIDK

SEQ ID NO: 110 - protein, 23 aa, Unknown
  Description of Unknown: FLT3 peptide
FGKVLGSGAFGKVMNATAYGISK

SEQ ID NO: 111 - protein, 23 aa, Unknown
  Description of Unknown: PDGFRA peptide
LGRVLGSGAFGKVVEGTAYGLSR

SEQ ID NO: 112 - protein, 23 aa, Unknown
  Description of Unknown: ERBB3 peptide
KLKVLGSGVFGTVHKGVWIPEGE

SEQ ID NO: 113 - protein, 23 aa, Unknown
  Description of Unknown: ERBB4 peptide
RVKVLGSGAFGTVYKGIWVPEGE

SEQ ID NO: 114 - protein, 23 aa, Unknown
  Description of Unknown: JAK2 peptide
FLQQLGKGNFGSVEMCRYDPLQD

SEQ ID NO: 115 - protein, 23 aa, Unknown
  Description of Unknown: ROS1 peptide
LRLLLGSGAFGEVYEGTAVDILG

SEQ ID NO: 116 - DNA, 22 bp, Unknown
  Description of Unknown: DDR2 oligonucleotide
tcagtttctttcccgccacgag

SEQ ID NO: 117 - DNA, 22 bp, Unknown
  Description of Unknown: DDR2 oligonucleotide
tcagtttctttyccgccacgag

SEQ ID NO: 118 - DNA, 22 bp, Unknown
  Description of Unknown: DDR2 oligonucleotide
tcagtttcttttccgccacgag

SEQ ID NO: 119 - DNA, 22 bp, Unknown
  Description of Unknown: DDR2 oligonucleotide
tcagtttttttcccgccacgag

SEQ ID NO: 120 - protein, 8 aa, Unknown
  Description of Unknown: DDR2 peptide
NQFLSRHE

SEQ ID NO: 121 - protein, 17 aa, Unknown
  Description of Unknown: DDR2 peptide
YMENGDLNQFLSRHEPP

SEQ ID NO: 122 - protein, 17 aa, Unknown
  Description of Unknown: BRAF peptide
WCKGSSLYHHLHIIETK

SEQ ID NO: 123 - protein, 17 aa, Unknown
  Description of Unknown: EGFR peptide
LMPFGCLLDYVREHKDN

SEQ ID NO: 124 - protein, 17 aa, Unknown
  Description of Unknown: ERBB2 peptide
LMPYGCLLDHVRENRGR

SEQ ID NO: 125 - protein, 16 aa, Unknown
  Description of Unknown: ABL1 peptide
FNTYGNLLDYLRECNR

SEQ ID NO: 126 - protein, 17 aa, Unknown
  Description of Unknown: ALK peptide
LMAGGDLKSFLRETRPR

SEQ ID NO: 127 - protein, 16 aa, Unknown
  Description of Unknown: AKT1 peptide
YANGGELFFHLSRERV

SEQ ID NO: 128 - protein, 17 aa, Unknown
  Description of Unknown: MET peptide
YMKHGDLRNFIRNETHN

SEQ ID NO: 129 - protein, 17 aa, Unknown
  Description of Unknown: FGFR1 peptide
YASKGNLREYLQARRPP

SEQ ID NO: 130 - protein, 17 aa, Unknown
  Description of Unknown: FGFR2 peptide
YASKGNLREYLRARRPP

SEQ ID NO: 131 - protein, 17 aa, Unknown
  Description of Unknown: FGFR3 peptide
YASKGNLREYLRARRPP

SEQ ID NO: 132 - protein, 17 aa, Unknown
  Description of Unknown: FLT3 peptide
YCCYGDLLNYLRSKREK

SEQ ID NO: 133 - protein, 17 aa, Unknown
  Description of Unknown: PDGFRA peptide
YCFYGDLVNYLHKNRDS

SEQ ID NO: 134 - protein, 17 aa, Unknown
  Description of Unknown: ERBB3 peptide
YLPLGSLLDHVRQHRGA

SEQ ID NO: 135 - protein, 17 aa, Unknown
  Description of Unknown: ERBB4 peptide
LMPHGCLLEYVHEHKDN

SEQ ID NO: 136 - protein, 17 aa, Unknown
  Description of Unknown: JAK2 peptide
YLPYGSLRDYLQKHKER

SEQ ID NO: 137 - protein, 17 aa, Unknown
  Description of Unknown: ROS1 peptide
LMEGGDLLTYLRKARMA

SEQ ID NO: 138 - DNA, 22 bp, Unknown
  Description of Unknown: DDR2 oligonucleotide
gcatgaagtacctttcctctct

SEQ ID NO: 139 - DNA, 22 bp, Unknown
  Description of Unknown: DDR2 oligonucleotide
gcatgaagtacytttcctctct

SEQ ID NO: 140 - DNA, 22 bp, Unknown
  Description of Unknown: DDR2 oligonucleotide
gcatgaagtacttttcctctct

SEQ ID NO: 141 - DNA, 21 bp, Unknown
  Description of Unknown: DDR2 oligonucleotide
gcatgaagtactttcctctct

SEQ ID NO: 142 - DNA, 20 bp, Unknown
  Description of Unknown: DDR2 oligonucleotide
gcatgaagtacctttcctct

SEQ ID NO: 143 - protein, 7 aa, Unknown
  Description of Unknown: DDR2 peptide
GMKYLSS

SEQ ID NO: 144 - protein, 37 aa, Unknown
  Description of Unknown: DDR2 polypeptide
VSYTNLKFMATQIASGMKYLSSLNFVHRDLATRNCLV

SEQ ID NO: 145 - protein, 37 aa, Unknown
  Description of Unknown: BRAF polypeptide
FEMIKLIDIARQTAQGMDYLHAKSIIHRDLKSNNIFL

SEQ ID NO: 146 - protein, 37 aa, Unknown
  Description of Unknown: EGFR polypeptide
IGSQYLLNWCVQIAKGMNYLEDRRLVHRDLAARNVLV

SEQ ID NO: 147 - protein, 37 aa, Unknown
  Description of Unknown: ERBB2 polypeptide
LGSQDLLNWCMQIAKGMSYLEDVRLVHRDLAARNVLV

SEQ ID NO: 148 - protein, 37 aa, Unknown
  Description of Unknown: ABL1 polypeptide
VNAVVLLYMATQISSAMEYLEKKNFIHRDLAARNCLV

SEQ ID NO: 149 - protein, 37 aa, Unknown
  Description of Unknown: ALK polypeptide
LAMLDLLHVARDIACGCQYLEENHFIHRDIAARNCLL

SEQ ID NO: 150 - protein, 38 aa, Unknown
  Description of Unknown: AKT1 polypeptide
FSEDRARFYGAEIVSALDYLHSEKNVVYRDLKLENLML

SEQ ID NO: 151 - protein, 37 aa, Unknown
  Description of Unknown: MET polypeptide
PTVKDLIGFGLQVAKGMKYLASKKFVHRDLAARNCML

SEQ ID NO: 152 - protein, 37 aa, Unknown
  Description of Unknown: FGFR1 polypeptide
LSSKDLVSCAYQVARGMEYLASKKCIHRDLAARNVLV

SEQ ID NO: 153 - protein, 37 aa, Unknown
  Description of Unknown: FGFR2 polypeptide
MTFKDLVSCTYQVARGMEYLASQKCIHRDLAARNVLV

SEQ ID NO: 154 - protein, 37 aa, Unknown
  Description of Unknown: FGFR3 polypeptide
LTFKDLVSCAYQVARGMEYLASQKCIHRDLAARNVLV

SEQ ID NO: 155 - protein, 37 aa, Unknown
  Description of Unknown: FLT3 polypeptide
LTFEDLLCFAYQVAKGMEFLEFKSCVHRDLAARNVLV

SEQ ID NO: 156 - protein, 37 aa, Unknown
  Description of Unknown: PDGFRA polypeptide
LTLLDLLSFTYQVARGMEFLASKNCVHRDLAARNVLL

SEQ ID NO: 157 - protein, 37 aa, Unknown
  Description of Unknown: ERBB3 polypeptide
LGPQLLLNWGVQIAKGMYYLEEHGMVHRNLAARNVLL

SEQ ID NO: 158 - protein, 37 aa, Unknown
  Description of Unknown: ERBB4 polypeptide
IGSQLLLNWCVQIAKGMMYLEERRLVHRDLAARNVLV

SEQ ID NO: 159 - protein, 37 aa, Unknown
  Description of Unknown: JAK2 polypeptide
IDHIKLLQYTSQICKGMEYLGTKRYIHRDLATRNILV

SEQ ID NO: 160 - protein, 37 aa, Unknown
  Description of Unknown: ROS1 polypeptide
LTLVDLVDLCVDISKGCVYLERMHFIHRDLAARNCLV

SEQ ID NO: 161 - DNA, 84 bp, Unknown
  Description of Unknown: DDR2 oligonucleotide
acaccaatctgaagtttatggctacccaaattgcctctggcatgaagtacctttyctctcttaattttgttcaccgagatctgg

SEQ ID NO: 162 - DNA, 84 bp, Unknown
  Description of Unknown: DDR2 oligonucleotide
acaccaatctgaagtttatggctacccaaattgcctctggcatgaagtacctttcctctcttaattttgttcaccgagatctgg

SEQ ID NO: 163 - protein, 28 aa, Unknown
  Description of Unknown: DDR2 peptide
YTNLKFMATQIASGMKYLSSLNFVHRDL

SEQ ID NO: 164 - DNA, 81 bp, Unknown
  Description of Unknown: DDR2 oligonucleotide
gtgctggatggaaatagtaamccctatgacattttcctaaaggacttggagccgcccattgtagccagatttgtccggttc

SEQ ID NO: 165 - DNA, 81 bp, Unknown
  Description of Unknown: DDR2 oligonucleotide
gtgctggatggaaatagtaacccctatgacattttcctaaaggacttggagccgcccattgtagccagatttgtccggttc

SEQ ID NO: 166 - protein, 27 aa, Unknown
  Description of Unknown: DDR2 peptide
VLDGNSNPYDIFLKDLEPPIVARFVRF

SEQ ID NO: 167 - DNA, 81 bp, Unknown
  Description of Unknown: DDR2 oligonucleotide
gatccaatgcttaaagttgatgacagcaacactcrgatcctgattggctgcttggtggccatcatctttatcctcctggcc

SEQ ID NO: 168 - DNA, 81 bp, Unknown
  Description of Unknown: DDR2 oligonucleotide
gatccaatgcttaaagttgatgacagcaacactcggatcctgattggctgcttggtggccatcatctttatcctcctggcc

SEQ ID NO: 169 - protein, 27 aa, Unknown
  Description of Unknown: DDR2 peptide
DPMLKVDDSNTRILIGCLVAIIFILLA